European Patent Application EP 4 166 573 A1, published April 19, 2023. Title: INSULIN DEGLUDEC DERIVATIVE, PREPARATION METHOD THEREFOR, AND APPLICATION THEREOF. Applicant: NINGBO KUNPENG BIOTECH CO., LTD. The sequence listing filed with the application follows.

SEQUENCE LISTING (22 sequences)

SEQ ID NO: 1 - protein, 105 aa, Artificial Sequence
  Insulin degludec fusion protein
MVSKGEELFTGVKLTLKFICTTYVQERTISFKDTYKTRAEVKFEGDENLYFQGRFVNQHLCGSHLVEALYLVCGERGFFYTPKRGIVEQCCTSICSLYQLENYCN

SEQ ID NO: 2 - protein, 29 aa, Artificial Sequence
  B chain of insulin degludec
FVNQHLCGSHLVEALYLVCGERGFFYTPK

SEQ ID NO: 3 - protein, 21 aa, Artificial Sequence
  A chain of insulin degludec
GIVEQCCTSICSLYQLENYCN

SEQ ID NO: 4 - protein, 6 aa, Artificial Sequence
  linker peptide
RRGSKR

SEQ ID NO: 5 - protein, 6 aa, Artificial Sequence
  linker peptide
RRAAKR

SEQ ID NO: 6 - protein, 9 aa, Artificial Sequence
  linker peptide
RRYPGDVKR

SEQ ID NO: 7 - protein, 35 aa, Artificial Sequence
  linker peptide
RREAEDLQVGQVELGGGPGAGSLQPLALEGSLQKR

SEQ ID NO: 8 - protein, 12 aa, Artificial Sequence
  leader peptide
MVSKGEELFTGV

SEQ ID NO: 9 - protein, 34 aa, Artificial Sequence
  green fluorescent protein folding unit
KLTLKFICTTYVQERTISFKDTYKTRAEVKFEGD

SEQ ID NO: 10 - protein, 7 aa, Artificial Sequence
  Restriction site of TEV enzyme
ENLYFQG

SEQ ID NO: 11 - protein, 13 aa, Artificial Sequence
  β-folding unit
VPILVELDGDVNG

SEQ ID NO: 12 - protein, 14 aa, Artificial Sequence
  β-folding unit
HKFSVRGEGEGDAT

SEQ ID NO: 13 - protein, 10 aa, Artificial Sequence
  β-folding unit
KLTLKFICTT

SEQ ID NO: 14 - protein, 11 aa, Artificial Sequence
  β-folding unit
YVQERTISFKD

SEQ ID NO: 15 - protein, 13 aa, Artificial Sequence
  β-folding unit
TYKTRAEVKFEGD

SEQ ID NO: 16 - protein, 13 aa, Artificial Sequence
  β-folding unit
TLVNRIELKGIDF

SEQ ID NO: 17 - protein, 10 aa, Artificial Sequence
  β-folding unit
HNVYITADKQ

SEQ ID NO: 18 - protein, 14 aa, Artificial Sequence
  β-folding unit
GIKANFKIRHNVED

SEQ ID NO: 19 - protein, 14 aa, Artificial Sequence
  β-folding unit
VQLADHYQQNTPIG

SEQ ID NO: 20 - protein, 12 aa, Artificial Sequence
  β-folding unit
HYLSTQSVLSKD

SEQ ID NO: 21 - protein, 13 aa, Artificial Sequence
  β-folding unit
HMVLLEFVTAAGI

SEQ ID NO: 22 - protein, 103 aa, Artificial Sequence
  Fusion protein
MKKLLFAIPLVVPFYSHSTMELEICSWYHMGIRSFLEQKLISEEDLNSAVDRFVNQHLCGSHLVEALYLVCGERGFFYTPKRGIVEQCCTSICSLYQLENYCN